European Patent Specification EP 3 491 022 B1, published September 10, 2025. Title: ANTIBODIES TARGETING TUMOR ASSOCIATED MACROPHAGES AND USES THEREOF. Applicant: INSERM. The sequence listing filed with the application follows.

SEQUENCE LISTING (16 sequences)

SEQ ID NO: 1 - protein, 8 aa, Artificial Sequence
  H-CDR1
GFSLTGYG

SEQ ID NO: 2 - protein, 7 aa, Artificial Sequence
  H-CDR2
IWGDGST

SEQ ID NO: 3 - protein, 9 aa, Artificial Sequence
  H-CDR3
ARDLKFAYW

SEQ ID NO: 4 - protein, 6 aa, Artificial Sequence
  L-CDR1
QHVTTA

SEQ ID NO: 5 - protein, 3 aa, Artificial
  L-CDR2
SAS

SEQ ID NO: 6 - protein, 9 aa, Artificial Sequence
  L-CDR3
QQHYTTPWT

SEQ ID NO: 7 - protein, 114 aa, Artificial Sequence
  H-VD
QVQLKESGPGLVAPSQSLSITCTVSGFSLTGYGVNWVRQPPGKGLEWLGMIWGDGSTDYNSDLKSRLSITEDNSKRQVFLKMDSLQTEDTARYYCARDLKFAYWGQGTLVTVSA

SEQ ID NO: 8 - protein, 107 aa, Artificial Sequence
  L-VD
DIVMTQSHKFMSSSVGDRVSITCKASQHVTTAVAWFQQKPGQSPKLLIYSASFRYTGVPDRFTGSGSGTDFTFTISTVQAEDLAVYYCQQHYTTPWTFGGGTKLEIK

SEQ ID NO: 9 - DNA, 340 bp, Artificial Sequence
  H-VD nucleic acid sequence
caggtgcagctgaaggagtcaggacctggcctggtggcgccctcacagagcctgtccatcacatgcaccgtctcagggttctcattaaccggctatggtgtaaactgggttcgccagcctccaggaagggtctggagtggctgggaatgatatggggtgatggaagcacagactataattcagatctcaaatccagactgagcatcaccgaggacaactccaagcgccaagttttcttaaaaatggacagtctgaaactgaagacacagccaggtactactgtgccagagatcttaagtttgcttactggggccaagggactctggtcactgtctctgca

SEQ ID NO: 10 - DNA, 319 bp, Artificial Sequence
  L-VD nucleic acid sequence
gacattgtgatgacccagtctcacaaattcatgtcctcatcagtaggagacagggtcagcatcacctgcaaggccagtcaacatgtgactactgctgttgcctggtttcaacagaaaccaggacaattcctaaactactgatttactcggcatccttccggtacactggagtccctgatcgcttcactggcagtggatctgggacggatttcactttcaccatcagcactgtgcaggctgaagacctggcagttattactgtcagcaacattatactactccgtggacgttcggtggaggcaccaagctggaaatcaaa

SEQ ID NO: 11 - protein, 7 aa, Artificial Sequence
  H-CDR1 Kabat system
GFSLTGY

SEQ ID NO: 12 - protein, 5 aa, Artificial Sequence
  H-CDR2 Kabat system
WGDGS

SEQ ID NO: 13 - protein, 6 aa, Artificial Sequence
  H-CDR3 Kabat system
DLKFAY

SEQ ID NO: 14 - protein, 11 aa, Artificial Sequence
  L-CDR1 Kabat system
KASQHVTTAVA

SEQ ID NO: 15 - protein, 7 aa, Artificial Sequence
  L-CDR2 Kabat system
SASFRYT

SEQ ID NO: 16 - protein, 9 aa, Artificial Sequence
  L-CDR3 Kabat system
QQHYTTPWT